European Patent Application EP 4 177 273 A1, published May 10, 2023. Title: Combination Therapy Involving Antibodies Against Claudin 18.2 For Treatment Of Cancer. Applicant: Astellas Pharma Inc. Application EP, filed February 18, 2014. The sequence listing filed with the application follows.

SEQUENCE LISTING (54 sequences)

SEQ ID NO: 1 - protein, 261 aa, Homo sapiens
MAVTACQGLGFVVSLIGIAGIIAATCMDQWSTQDLYNNPVTAVFNYQGLWRSCVRESSGFTECRGYFTLLGLPAMLQAVRALMIVGIVLGAIGLLVSIFALKCIRIGSMEDSAKANMTLTSGIMFIVSGLCAIAGVSVFANMLVTNFWMSTANMYTGMGGMVQTVQTRYTFGAALFVGWVAGGLTLIGGVMMCIACRGLAPEETNYKAVSYHASGHSVAYKPGGFKASTGFGSNTKNKKIYDGGARTEDEVQSYPSKHDYV

SEQ ID NO: 2 - protein, 261 aa, Homo sapiens
MSTTTCQVVAFLLSILGLAGCIAATGMDMWSTQDLYDNPVTSVFQYEGLWRSCVRQSSGFTECRPYFTILGLPAMLQAVRALMIVGIVLGAIGLLVSIFALKCIRIGSMEDSAKANMTLTSGIMFIVSGLCAIAGVSVFANMLVTNFWMSTANMYTGMGGMVQTVQTRYTFGAALFVGWVAGGLTLIGGVMMCIACRGLAPEETNYKAVSYHASGHSVAYKPGGFKASTGFGSNTKNKKIYDGGARTEDEVQSYPSKHDYV

SEQ ID NO: 3 - protein, 10 aa, Homo sapiens
DQWSTQDLYN

SEQ ID NO: 4 - protein, 11 aa, Homo sapiens
NNPVTAVFNYQ

SEQ ID NO: 5 - protein, 14 aa, Homo sapiens
STQDLYNNPVTAVF

SEQ ID NO: 6 - protein, 13 aa, Homo sapiens
TNFWMSTANMYTG

SEQ ID NO: 7 - protein, 13 aa, Homo sapiens
DSAKANMTLTSGI

SEQ ID NO: 8 - protein, 55 aa, Homo sapiens
MDQWSTQDLYNNPVTAVFNYQGLWRSCVRESSGFTECRGYFTLLGLPAMLQAVRA

SEQ ID NO: 9 - protein, 24 aa, Homo sapiens
FALKCIRIGSMEDSAKANMTLTSG

SEQ ID NO: 10 - protein, 40 aa, Homo sapiens
ANMLVTNFWMSTANMYTGMGGMVQTVQTRYTFGAALFVGW

SEQ ID NO: 11 - protein, 153 aa, Homo sapiens
MDQWSTQDLYNNPVTAVFNYQGLWRSCVRESSGFTECRGYFTLLGLPAMLQAVRALMIVGIVLGAIGLLVSIFALKCIRIGSMEDSAKANMTLTSGIMFIVSGLCAIAGVSVFANMLVTNFWMSTANMYTGMGGMVQTVQTRYTFGAALFVGW

SEQ ID NO: 12 - protein, 107 aa, synthetic construct [sequence omitted]

SEQ ID NO: 13 - protein, 326 aa, synthetic construct
  REGION 1..326: note = Description of artificial sequence: Translation of PCR product
GPSVFPLAPSSKSTSGGTAALGCLVKDYFPEPVTVSWNSGALTSGVHTFPAVLQSSGLYSLSSVVTVPSSSLGTQTYICNVNHKPSNTKVDKKVEPKSCDKTHTCPPCPAPELLGGPSVFLFPPKPKDTLMISRTPEVTCVVVDVSHEDPEVKFNWYVDGVEVHNAKTKPREEQYNSTYRVVSVLTVLHQDWLNGKEYKCKVSNKALPAPIEKTISKAKGQPREPQVYTLPPSRDELTKNQVSLTCLVKGFYPSDIAVEWESNGQPENNYKTTPPVLDSDGSFFLYSKLTVDKSRWQQGNVFSCSVMHEALHNHYTQKSLSLSPGK

SEQ ID NO: 14 - protein, 466 aa, synthetic construct
  REGION 1..466: note = Description of artificial sequence: chimeric monoclonal antibody
MEWTWVFLFLLSVTAGVHSQVQLQQSGAELMKPGASVKISCKATGYTFSSYWIEWVKQRPGHGLEWIGEILPGSGSTNYNEKFKGKATFTADTSSNTAYMQLSSLTSEDSAVYYCARYDYPWFAYWGQGTLVTVSAASTKGPSVFPLAPSSKSTSGGTAALGCLVKDYFPEPVTVSWNSGALTSGVHTFPAVLQSSGLYSLSSVVTVPSSSLGTQTYICNVNHKPSNTKVDKKVEPKSCDKTHTCPPCPAPELLGGPSVFLFPPKPKDTLMISRTPEVTCVVVDVSHEDPEVKFNWYVDGVEVHNAKTKPREEQYNSTYRVVSVLTVLHQDWLNGKEYKCKVSNKALPAPIEKTISKAKGQPREPQVYTLPPSRDELTKNQVSLTCLVKGFYPSDIAVEWESNGQPENNYKTTPPVLDSDGSFFLYSKLTVDKSRWQQGNVFSCSVMHEALHNHYTQKSLSLSPGK

SEQ ID NO: 15 - protein, 467 aa, synthetic construct
  REGION 1..467: note = Description of artificial sequence: chimeric monoclonal antibody
MDWLWNLLFLMAAAQSIQAQIQLVQSGPELKKPGETVKISCKASGYTFTNYGMNWVKQAPGKGLKWMGWINTNTGEPTYAEEFKGRFAFSLETSASTAYLQINNLKNEDTATYFCARLGFGNAMDYWGQGTSVTVSSASTKGPSVFPLAPSSKSTSGGTAALGCLVKDYFPEPVTVSWNSGALTSGVHTFPAVLQSSGLYSLSSVVTVPSSSLGTQTYICNVNHKPSNTKVDKKVEPKSCDKTHTCPPCPAPELLGGPSVFLFPPKPKDTLMISRTPEVTCVVVDVSHEDPEVKFNWYVDGVEVHNAKTKPREEQYNSTYRVVSVLTVLHQDWLNGKEYKCKVSNKALPAPIEKTISKAKGQPREPQVYTLPPSRDELTKNQVSLTCLVKGFYPSDIAVEWESNGQPENNYKTTPPVLDSDGSFFLYSKLTVDKSRWQQGNVFSCSVMHEALHNHYTQKSLSLSPGK

SEQ ID NO: 16 - protein, 465 aa, synthetic construct
  REGION 1..465: note = Description of artificial sequence: chimeric monoclonal antibody
MEWIWIFLFILSGTAGVHSQVQLQQSGAELARPGASVKLSCKASGYTFTDYYINWVKQRTGQGLEWIGEIYPGSGNTYYNEKFKGKATLTADKSSSTAYMQLSSLTSEDSAVYFCARSYGAFDYWGQGTTLTVSSASTKGPSVFPLAPSSKSTSGGTAALGCLVKDYFPEPVTVSWNSGALTSGVHTFPAVLQSSGLYSLSSVVTVPSSSLGTQTYICNVNHKPSNTKVDKKVEPKSCDKTHTCPPCPAPELLGGPSVFLFPPKPKDTLMISRTPEVTCVVVDVSHEDPEVKFNWYVDGVEVHNAKTKPREEQYNSTYRVVSVLTVLHQDWLNGKEYKCKVSNKALPAPIEKTISKAKGQPREPQVYTLPPSRDELTKNQVSLTCLVKGFYPSDIAVEWESNGQPENNYKTTPPVLDSDGSFFLYSKLTVDKSRWQQGNVFSCSVMHEALHNHYTQKSLSLSPGK

SEQ ID NO: 17 - protein, 467 aa, synthetic construct
  REGION 1..467: note = Description of artificial sequence: chimeric monoclonal antibody
MGWSCIILFLVATATGVHSQVQLQQPGAELVRPGASVKLSCKASGYTFTSYWINWVKQRPGQGLEWIGNIYPSDSYTNYNQKFKDKATLTVDKSSSTAYMQLSSPTSEDSAVYYCTRSWRGNSFDYWGQGTTLTVSSASTKGPSVFPLAPSSKSTSGGTAALGCLVKDYFPEPVTVSWNSGALTSGVHTFPAVLQSSGLYSLSSVVTVPSSSLGTQTYICNVNHKPSNTKVDKKVEPKSCDKTHTCPPCPAPELLGGPSVFLFPPKPKDTLMISRTPEVTCVVVDVSHEDPEVKFNWYVDGVEVHNAKTKPREEQYNSTYRVVSVLTVLHQDWLNGKEYKCKVSNKALPAPIEKTISKAKGQPREPQVYTLPPSRDELTKNQVSLTCLVKGFYPSDIAVEWESNGQPENNYKTTPPVLDSDGSFFLYSKLTVDKSRWQQGNVFSCSVMHEALHNHYTQKSLSLSPGK

SEQ ID NO: 18 - protein, 466 aa, synthetic construct
  REGION 1..466: note = Description of artificial sequence: chimeric monoclonal antibody
MEWRIFLFILSGTAGVHSQVQLQQSGPELVKPGASVKMSCKASGYTFTDYVISWVKQRTGQGLEWIGEIYPGSGSTYYNEKFKGKATLTADKSSNTAYMQLSSLTSEDSAVYFCARGVLLRAMDYWGQGTSVTVSSASTKGPSVFPLAPSSKSTSGGTAALGCLVKDYFPEPVTVSWNSGALTSGVHTFPAVLQSSGLYSLSSVVTVPSSSLGTQTYICNVNHKPSNTKVDKKVEPKSCDKTHTCPPCPAPELLGGPSVFLFPPKPKDTLMISRTPEVTCVVVDVSHEDPEVKFNWYVDGVEVHNAKTKPREEQYNSTYRVVSVLTVLHQDWLNGKEYKCKVSNKALPAPIEKTISKAKGQPREPQVYTLPPSRDELTKNQVSLTCLVKGFYPSDIAVEWESNGQPENNYKTTPPVLDSDGSFFLYSKLTVDKSRWQQGNVFSCSVMHEALHNHYTQKSLSLSPGK

SEQ ID NO: 19 - protein, 469 aa, synthetic construct [sequence omitted]

SEQ ID NO: 20 - protein, 240 aa, synthetic construct
  REGION 1..240: note = Description of artificial sequence: chimeric monoclonal antibody
MESQTQVLMSLLFWVSGTCGDIVMTQSPSSLTVTAGEKVTMSCKSSQSLLNSGNQKNYLTWYQQKPGQPPKLLIYWASTRESGVPDRFTGSGSGTDFTLTISSVQAEDLAVYYCQNDYSYPLTFGAGTKLELKRTVAAPSVFIFPPSDEQLKSGTASVVCLLNNFYPREAKVQWKVDNALQSGNSQESVTEQDSKDSTYSLSSTLTLSKADYEKHKVYACEVTHQGLSSPVTKSFNRGEC

SEQ ID NO: 21 - protein, 235 aa, synthetic construct
  REGION 1..235: note = Description of artificial sequence: chimeric monoclonal antibody
MHFQVQIFSFLLISASVIMSRGQIVLTQSPAIMSASPGEKVTITCSASSSVSYMHWFQQKPGTSPKLWIYSTSNLASGVPARFSGSGSGTSYSLTISRMEAEDAATYYCQQRSSYPPTFGGGTKLEIKRTVAAPSVFIFPPSDEQLKSGTASVVCLLNNFYPREAKVQWKVDNALQSGNSQESVTEQDSKDSTYSLSSTLTLSKADYEKHKVYACEVTHQGLSSPVTKSFNRGEC

SEQ ID NO: 22 - protein, 234 aa, synthetic construct
  REGION 1..234: note = Description of artificial sequence: chimeric monoclonal antibody
MEFQTQVFVFVLLWLSGVDGDIVMTQSQKFMSTSVGDRVSITCKASQNVRTAVAWYQQKPGQSPKALIYLASNRHTGVPDRFTGSGSGTDFTLTISNVQSEDLADYFCLQHWNYPLTFGGGTKLEIKRTVAAPSVFIFPPSDEQLKSGTASVVCLLNNFYPREAKVQWKVDNALQSGNSQESVTEQDSKDSTYSLSSTLTLSKADYEKHKVYACEVTHQGLSSPVTKSFNRGEC

SEQ ID NO: 23 - protein, 240 aa, synthetic construct
  REGION 1..240: note = Description of artificial sequence: chimeric monoclonal antibody
MDSQAQVLMLLLLWVSGTCGDIVMSQSPSSLAVSVGEKVTMSCKSSQSLLYSSNQKNYLAWYQQKPGQSPKLLIYWASTRESGVPDRFTGSGSGTDFTLTISSVKAEDLAVYYCQQYYSYPLTFGAGTKLELKRTVAAPSVFIFPPSDEQLKSGTASVVCLLNNFYPREAKVQWKVDNALQSGNSQESVTEQDSKDSTYSLSSTLTLSKADYEKHKVYACEVTHQGLSSPVTKSFNRGEC

SEQ ID NO: 24 - protein, 240 aa, synthetic construct
  REGION 1..240: note = Description of artificial sequence: chimeric monoclonal antibody
MESQTQVLMSLLFWVSGTCGDIVMTQSPSSLTVTAGEKVTMSCKSSQSLLNSGNQKNYLTWYQQKPGQPPKLLIYWASTRESGVPDRFTGSGSGTDFTLTISSVQAEDLAVYYCQNDYSYPFTFGSGTKLEIKRTVAAPSVFIFPPSDEQLKSGTASVVCLLNNFYPREAKVQWKVDNALQSGNSQESVTEQDSKDSTYSLSSTLTLSKADYEKHKVYACEVTHQGLSSPVTKSFNRGEC

SEQ ID NO: 25 - protein, 239 aa, synthetic construct
  REGION 1..239: note = Description of artificial sequence: chimeric monoclonal antibody
MDSQAQVLILLLLWVSGTCGDIVMSQSPSSLAVSAGEKVTMSCKSSQSLLNSRTRKNYLAWYQQKPGQSPKLLIYWASTRESGVPDRFTGSGSGTDFTLTISSVQAEDLAVYYCKQSYNLYTFGGGTKLEIKRTVAAPSVFIFPPSDEQLKSGTASVVCLLNNFYPREAKVQWKVDNALQSGNSQESVTEQDSKDSTYSLSSTLTLSKADYEKHKVYACEVTHQGLSSPVTKSFNRGEC

SEQ ID NO: 26 - protein, 240 aa, synthetic construct
  REGION 1..240: note = Description of artificial sequence: chimeric monoclonal antibody
MDSQAQVLMLLLLWVSGTCGDIVMSQSPSSLAVSVGEKVTMSCKSSQSLLYSSNQKNYLAWYQQKPGQSPKLLIYWASTRESGVPDRFTGSGSATDFTLTISSVQAEDLADYHCGQGYSYPYTFGGGTKLEIKRTVAAPSVFIFPPSDEQLKSGTASVVCLLNNFYPREAKVQWKVDNALQSGNSQESVTEQDSKDSTYSLSSTLTLSKADYEKHKVYACEVTHQGLSSPVTKSFNRGEC

SEQ ID NO: 27 - protein, 240 aa, synthetic construct; identical to SEQ ID NO: 23
  REGION 1..240: note = Description of artificial sequence: chimeric monoclonal antibody

SEQ ID NO: 28 - protein, 234 aa, synthetic construct
  REGION 1..234: note = Description of artificial sequence: chimeric monoclonal antibody
MESQTLVFISILLWLYGADGNIVMTQSPKSMSMSVGERVTLTCKASENVVTYVSWYQQKPEQSPKLLIYGASNRYTGVPDRFTGSGSATDFTLTISSVKAEDLAVYYCQQYYSYPLTFGAGTKLELKRTVAAPSVFIFPPSDEQLKSGTASVVCLLNNFYPREAKVQWKVDNALQSGNSQESVTEQDSKDSTYSLSSTLTLSKADYEKHKVYACEVTHQGLSSPVTKSFNRGEC

SEQ ID NO: 29 - protein, 117 aa, synthetic construct
  REGION 1..117: note = Description of artificial sequence: Translation of PCR product
QVQLQQSGAELMKPGASVKISCKATGYTFSSYWIEWVKQRPGHGLEWIGEILPGSGSTNYNEKFKGKATFTADTSSNTAYMQLSSLTSEDSAVYYCARYDYPWFAYWGQGTLVTVSA

SEQ ID NO: 30 - protein, 118 aa, synthetic construct
  REGION 1..118: note = Description of artificial sequence: Translation of PCR product
QIQLVQSGPELKKPGETVKISCKASGYTFTNYGMNWVKQAPGKGLKWMGWINTNTGEPTYAEEFKGRFAFSLETSASTAYLQINNLKNEDTATYFCARLGFGNAMDYWGQGTSVTVSS

SEQ ID NO: 31 - protein, 116 aa, synthetic construct
  REGION 1..116: note = Description of artificial sequence: Translation of PCR product
QVQLQQSGAELARPGASVKLSCKASGYTFTDYYINWVKQRTGQGLEWIGEIYPGSGNTYYNEKFKGKATLTADKSSSTAYMQLSSLTSEDSAVYFCARSYGAFDYWGQGTTLTVSS

SEQ ID NO: 32 - protein, 118 aa, synthetic construct
  REGION 1..118: note = Description of artificial sequence: Translation of PCR product
QVQLQQPGAELVRPGASVKLSCKASGYTFTSYWINWVKQRPGQGLEWIGNIYPSDSYTNYNQKFKDKATLTVDKSSSTAYMQLSSPTSEDSAVYYCTRSWRGNSFDYWGQGTTLTVSS

SEQ ID NO: 33 - protein, 118 aa, synthetic construct
  REGION 1..118: note = Description of artificial sequence: Translation of PCR product
QVQLQQSGPELVKPGASVKMSCKASGYTFTDYVISWVKQRTGQGLEWIGEIYPGSGSTYYNEKFKGKATLTADKSSNTAYMQLSSLTSEDSAVYFCARGVLLRAMDYWGQGTSVTVSS

SEQ ID NO: 34 - protein, 120 aa, synthetic construct
  REGION 1..120: note = Description of artificial sequence: Translation of PCR product
QVHLQQSGSELRSPGSSVKLSCKDFDSEVFPFAYMSWIRQKPGHGFEWIGDILPSIGRTIYGEKFEDKATLDADTVSNTAYLELNSLTSEDSAIYYCARGEGYGAWFAYWGQGTLVTVSA

SEQ ID NO: 35 - protein, 113 aa, synthetic construct
  REGION 1..113: note = Description of artificial sequence: Translation of PCR product
DIVMTQSPSSLTVTAGEKVTMSCKSSQSLLNSGNQKNYLTWYQQKPGQPPKLLIYWASTRESGVPDRFTGSGSGTDFTLTISSVQAEDLAVYYCQNDYSYPLTFGAGTKLELK

SEQ ID NO: 36 - protein, 106 aa, synthetic construct
  REGION 1..106: note = Description of artificial sequence: Translation of PCR product
QIVLTQSPAIMSASPGEKVTITCSASSSVSYMHWFQQKPGTSPKLWIYSTSNLASGVPARFSGSGSGTSYSLTISRMEAEDAATYYCQQRSSYPPTFGGGTKLEIK

SEQ ID NO: 37 - protein, 107 aa, synthetic construct
  REGION 1..107: note = Description of artificial sequence: Translation of PCR product
DIVMTQSQKFMSTSVGDRVSITCKASQNVRTAVAWYQQKPGQSPKALIYLASNRHTGVPDRFTGSGSGTDFTLTISNVQSEDLADYFCLQHWNYPLTFGGGTKLEIK

SEQ ID NO: 38 - protein, 113 aa, synthetic construct
  REGION 1..113: note = Description of artificial sequence: Translation of PCR product
DIVMSQSPSSLAVSVGEKVTMSCKSSQSLLYSSNQKNYLAWYQQKPGQSPKLLIYWASTRESGVPDRFTGSGSGTDFTLTISSVKAEDLAVYYCQQYYSYPLTFGAGTKLELK

SEQ ID NO: 39 - protein, 113 aa, synthetic construct
  REGION 1..113: note = Description of artificial sequence: Translation of PCR product
DIVMTQSPSSLTVTAGEKVTMSCKSSQSLLNSGNQKNYLTWYQQKPGQPPKLLIYWASTRESGVPDRFTGSGSGTDFTLTISSVQAEDLAVYYCQNDYSYPFTFGSGTKLEIK

SEQ ID NO: 40 - protein, 112 aa, synthetic construct
  REGION 1..112: note = Description of artificial sequence: Translation of PCR product
DIVMSQSPSSLAVSAGEKVTMSCKSSQSLLNSRTRKNYLAWYQQKPGQSPKLLIYWASTRESGVPDRFTGSGSGTDFTLTISSVQAEDLAVYYCKQSYNLYTFGGGTKLEIK

SEQ ID NO: 41 - protein, 113 aa, synthetic construct
  REGION 1..113: note = Description of artificial sequence: Translation of PCR product
DIVMSQSPSSLAVSVGEKVTMSCKSSQSLLYSSNQKNYLAWYQQKPGQSPKLLIYWASTRESGVPDRFTGSGSATDFTLTISSVQAEDLADYHCGQGYSYPYTFGGGTKLEIK

SEQ ID NO: 42 - protein, 113 aa, synthetic construct; identical to SEQ ID NO: 38
  REGION 1..113: note = Description of artificial sequence: Translation of PCR product

SEQ ID NO: 43 - protein, 107 aa, synthetic construct
  REGION 1..107: note = Description of artificial sequence: Translation of PCR product
NIVMTQSPKSMSMSVGERVTLTCKASENVVTYVSWYQQKPEQSPKLLIYGASNRYTGVPDRFTGSGSATDFTLTISSVKAEDLAVYYCQQYYSYPLTFGAGTKLELK

SEQ ID NO: 44 - protein, 15 aa, synthetic construct
  REGION 1..15: note = Epitope
MDQWSTQDLYNNPVT

SEQ ID NO: 45 - protein, 15 aa, synthetic construct
  REGION 1..15: note = Epitope
STQDLYNNPVTAVFN

SEQ ID NO: 46 - protein, 15 aa, synthetic construct
  REGION 1..15: note = Epitope
LYNNPVTAVFNYQGL

SEQ ID NO: 47 - protein, 15 aa, synthetic construct
  REGION 1..15: note = Epitope
PVTAVFNYQGLWRSC

SEQ ID NO: 48 - protein, 15 aa, synthetic construct
  REGION 1..15: note = Epitope
VFNYQGLWRSCVRES

SEQ ID NO: 49 - protein, 15 aa, synthetic construct
  REGION 1..15: note = Epitope
QGLWRSCVRESSGFT

SEQ ID NO: 50 - protein, 15 aa, synthetic construct
  REGION 1..15: note = Epitope
RSCVRESSGFTECRG

SEQ ID NO: 51 - DNA, 24 bp, synthetic construct
  misc_feature 1..24: note = Oligonucleotide
  source 1..24: mol_type = other DNA
agagagctctggcttcaccgagtg

SEQ ID NO: 52 - DNA, 26 bp, synthetic construct
  misc_feature 1..26: note = Oligonucleotide
  source 1..26: mol_type = other DNA
ccagaagttagtcaccagcatgttgg

SEQ ID NO: 53 - DNA, 25 bp, synthetic construct
  misc_feature 1..25: note = Oligonucleotide
  source 1..25: mol_type = other DNA
gggataatttcagctgactaaacag

SEQ ID NO: 54 - DNA, 25 bp, synthetic construct
  misc_feature 1..25: note = Oligonucleotide
  source 1..25: mol_type = other DNA
ttccgtttagttaggtgcagttatc